European Patent Application EP 4 209 577 A1, published July 12, 2023. Title: AGENT FOR INCREASING IgA ANTIBODY CONTENT IN BREAST FLUID. Applicant: Tohoku University The University of Tokyo. The sequence listing filed with the application follows.

SEQUENCE LISTING (19 sequences)

SEQ ID NO: 1 - DNA, 1968 bp, Bacteroides sp.
  misc_feature: Inventor:NOCHI Tomonori; USAMI Katsuki; ASO Hisashi; KIYONO Hiros hi; FUJIHASHI Kohtaro; SATO Shintaro
  misc_feature: 16S rRNA gene of the present Bacteroides bacteria strain
gtttgatcctggctcaggatgaacgctagctacaggcttaacacatgcaagtcgaggggcagcatgaaagtttgtttgcaaacttttgatggcgaccggcgcacgggtgagtaacacgtatccaacccgcctcatactcggggatagcctttcgaaagaaagattaatacccgatgtcatagtcctaccgcatgatgggactattaaagaatttcggtatgggatggggatgcgttccattagttagttggcggggtaacggcccaccaagacaacgatggataggggttctgagaggaaggtcccccacattggaactgagacacggtccaaactcctacgggaggcagcagtgaggaatattggtcaatggacgagagtctgaaccagccaagtagcgtgaaggatgactgccctatgggtttaaacttcttttatatgggaataaaacgttcacgtgtgggattttgtatgtaccatatgaataaggatcggctaactccgtgccagcagccgcggtaatacggaggatccgagcgttatccggatttattgggtttaaagggagcgtaggtggattgttaagtcagttgtgaaagtttgcggctcaaccgtaaaattgcagttgaaactggcagtcttgagtacagtagaggtgggcggaattcgtggtgtagcggtgaaatgcttagatatcacgaagaactccgattgcgaaggcagctcactggactgcaactgacactgaggctcgaaagtgtgggtatcaaacaggattagataccctggtagtccacacagtaaacgatgaatactcgctgtttgcgatatacagtaagcggccaagcgaaagcattaagtattccacctggggagtacgccggcaacggtgaaactcaaaggaattgacgggggcccgcacaagcggaggaacatgtggtttaattcgatgatacgcgaggaaccttacccgggcttaaattgcacctgaataatgtggaaacatgttagccgtaaggcaggtgtgaaggtgctgcatggttgtcgtcagctcgtgccgtgaggtgtcggcttaagtgccataacgagcgcaacccttatcttcagttactaacaggtcatgctgaggactctggagagactgccgtcgtaagatgtgaggaaggtggggatgacgtcaaatcagcacggcccttacgtccggggctacacacgtgttacaatgggaggtacagaaggccgctacctggcgacaggatgccaatccccaaaacctctctcagttcggatcgaagtctgcaacccgacttcgtgaagctggattcgctagtaatcgcgcatcagccatggcgcggtgaatacgttcccgggccttgtacacaccgcccgtcaagccatgaaagccgggggtacctgaagtacgtaaccgcaaggatcgtcctagggtaaaactggtaattggggctaagtcgtaacaaggtagccgtaccggaaggtgcggctggaacacctcctttctggagcgatgtcgtaacgatgactttttcaaggttctgttttttgtactactggtacttgtttatttataaaatatagaatcaaccatctatagaaagtatagaatagagataaacaagaagaaaacagaagccgagtctaactcaacaggtaaacaaggttgaactagtcctatagctcagttggttagagcgctacactgataatgtaaaggtcggcagttcaactctgcctgggactactccgaaactctttggggggattagctcagctggctaaagcatctgccttgcacgcagagggtcaacggttcgaatccgttattctccacagtctctgaaaagagaaacgatctttgacatgatgtaaccaaaaagtaaaaattttagtaaagagctaaaagtatataatcgaaccgtacgttcttgacgtatcaagactgtgtaacca

SEQ ID NO: 2 - DNA, 1493 bp, Prevotella sp.
  misc_feature: 16S rRNA gene of the present Prevotella bacteria strain
agagtttgatcctggctcaggatgaacgctagctacaggcttaacacatgcaagtcgcagggtaacgtgagggaagcttgcttcccttgacgacgactggcgcacgggtgagtaacgcgtatccaaccttcccatgaccacgggataacccgttgaaagacggactaataccgtatgacgtcgtttgctgacatcaaataacgattaaaggtttagcggtgatggatggggatgcgtctgattagcttgttggcggggtaacggcccaccaaggcgacgatcagtaggggttctgagaggaaggtcccccacattggaactgagacacggtccaaactcctacgggaggcagcagtgaggaatattggtcaatgggcgagagcctgaaccagccaagtagcgtgcaggatgacggccctatgggttgtaaactgcttttatgcggggataaagtgcgcgacgtgtcgtgcattgcaggtaccgcatgaataaggaccggctaattccgtgccagcagccgcggtaatacggaaggtccgggcgttatccggatttattgggtttaaagggagcgtaggccgccaggtaagcgtgttgtgaaatgtaccggctcaaccggtgaattgcagcgcgaactgtctggcttgagtgcacggtaagcaggcggaattcatggtgtagcggtgaaatgcttagatatcatgaagaactccgattgcgaaggcagcttgctgcagtgcgactgacgctgatgctcgaaggtgcgggtatcaaacaggattagataccctggtagtccgcacggtaaacgatggatgcccgctgtccgcccttttgtggcgggtggccaagcgaaagcgttaagcatcccacctggggagtacgccggcaacggtgaaactcaaaggaattgacgggggcccgcacaagcggaggaacatgtggtttaattcgatgatacgcgaggaaccttacccgggcttgaactgccagtgaacgatacagagatgttgaggcccttcggggcgctggtggaggtgctgcatggttgtcgtcagctcgtgccgtgaggtgtcggcttaagtgccataacgagcgcaaccccttttttcagttgccatcaggtaatgctgggcactctggagatactgccaccgcaaggtgtgaggaaggtggggatgacgtcaaatcagcacggcccttacgtccggggctacacacgtgttacaatggggcatacagagtgttggcttaacgcaagtttggtctaatcttcaaagtgtctcccagttcggactggggtctgcaacccgaccccacgaagctggattcgctagtaatcgcgcatcagccatggcgcggtgaatacgttcccgggccttgtacacaccgcccgtcaagccatgaaagccgggggtgcctgaagtccgtaaccgtcaaggagcggcctagggcaaaactggtgattggggctaagtcgtaacaaggtaacc

SEQ ID NO: 3 - DNA, 27 bp, Artificial
  Primer 1
tagttcattgctgctcctagtctcagc

SEQ ID NO: 4 - DNA, 27 bp, Artificial
  Primer 2
tgggatttgcatgcacagacgctgggg

SEQ ID NO: 5 - DNA, 29 bp, Artificial
  Primer 3
cttatttatactcccgcgctcactggagg

SEQ ID NO: 6 - DNA, 27 bp, Artificial
  Primer 4
ctaaagcgcatgctccagactgccttg

SEQ ID NO: 7 - DNA, 28 bp, Artificial
  Primer 5
gaggcaagaggactgccactagcttgag

SEQ ID NO: 8 - DNA, 30 bp, Artificial
  Forward probe
ggtagacagacttctagacttggtcaaccc

SEQ ID NO: 9 - DNA, 28 bp, Artificial
  Reverse probe
gtttagccttgaccacatggacatctgg

SEQ ID NO: 10 - DNA, 37 bp, Artificial
  Forward primer No.1 of mixture
  misc_feature (18)..(20): n stands for any base
  misc_feature (29)..(29): n stands for any base
tgctcttccgatctgacnnncctacgggnggcwgcag

SEQ ID NO: 11 - DNA, 38 bp, Artificial
  Forward primer No.2 of mixture
  misc_feature (18)..(21): n stands for any base
  misc_feature (30)..(30): n stands for any base
tgctcttccgatctgacnnnncctacgggnggcwgcag

SEQ ID NO: 12 - DNA, 39 bp, Artificial
  Forward primer No.3 of mixture
  misc_feature (18)..(22): n stands for any base
  misc_feature (31)..(31): n stands for any base
tgctcttccgatctgacnnnnncctacgggnggcwgcag

SEQ ID NO: 13 - DNA, 40 bp, Artificial
  Forward primer No.4 of mixture
  misc_feature (18)..(23): n stands for any base
  misc_feature (32)..(32): n stands for any base
tgctcttccgatctgacnnnnnncctacgggnggcwgcag

SEQ ID NO: 14 - DNA, 41 bp, Artificial
  Reverse primer No.1 of mixture
  misc_feature (18)..(20): n stands for any base
cgctcttccgatctctgnnngactachvgggtatctaatcc

SEQ ID NO: 15 - DNA, 42 bp, Artificial
  Reverse primer No.2 of mixture
  misc_feature (18)..(21): n stands for any base
cgctcttccgatctctgnnnngactachvgggtatctaatcc

SEQ ID NO: 16 - DNA, 43 bp, Artificial
  Reverse primer No.3 of mixture
  misc_feature (18)..(22): n stands for any base
cgctcttccgatctctgnnnnngactachvgggtatctaatcc

SEQ ID NO: 17 - DNA, 44 bp, Artificial
  Reverse primer No.4 of mixture
  misc_feature (18)..(23): n stands for any base
cgctcttccgatctctgnnnnnngactachvgggtatctaatcc

SEQ ID NO: 18 - DNA, 67 bp, Artificial
  Forward primer for second PCR
  misc_feature (25)..(30): n stands for any base
caagcagaagacggcatacgagatnnnnnngtgactggagttcagacgtgtgctcttccgatctgac

SEQ ID NO: 19 - DNA, 61 bp, Artificial
  Reverse primer for second PCR
aatgatacggcgaccaccgagatctacactctttccctacacgacgctcttccgatctctg